European Patent Application EP 4 450 627 A1, published October 23, 2024. Title: humanized anti-DNAM-1 antibody. Applicant: University of Tsukuba. The sequence listing filed with the application follows.

SEQUENCE LISTING (38 sequences)

SEQ ID NO: 1 - protein, 7 aa, Artificial sequence
  HCDR1 of hTKB1,hAKB1-A and hAKB1-B
SGYYWNW

SEQ ID NO: 2 - protein, 16 aa, Artificial sequence
  HCDR2 of hTKB1,hAKB1-A and hAKB1-B
YISYDGSNNYNPSLKN

SEQ ID NO: 3 - protein, 12 aa, Artificial sequence
  HCDR3 of hTKB1,hAKB1-A and hAKB1-B
AYYGNYVGYFDV

SEQ ID NO: 4 - protein, 11 aa, Artificial sequence
  LCDR1 of hTKB1,hAKB1-A and hAKB1-B
KASQSVSNDVA

SEQ ID NO: 5 - protein, 7 aa, Artificial sequence
  LCDR2 of hTKB1,hAKB1-A and hAKB1-B
YASNRYT

SEQ ID NO: 6 - protein, 9 aa, Artificial sequence
  LCDR3 of hTKB1,hAKB1-A and hAKB1-B
QQDYSSPLT

SEQ ID NO: 7 - protein, 121 aa, Mus musculus
DVQLQESGPGLVKPSQSLSLTCSVTGYSITSGYYWNWIRQFPGNKLEWMGYISYDGSNNYNPSLKNRISITRDTSKNQFFLKLNSVTTEDTATYYCARAYYGNYVGYFDVWGAGTTVTVSS

SEQ ID NO: 8 - protein, 110 aa, Mus musculus
SIVMTQTPKFLLVSAGDRVTITCKASQSVSNDVAWYQQKPGQSPKLLIYYASNRYTGVPDRFTGSGYGTDFTFTISTVQAEDLAVYFCQQDYSSPLTFGAGTKLELKRTV

SEQ ID NO: 9 - protein, 121 aa, Artificial sequence
  heavy chain variable region of hAKB1 VH1
QVQLQESGPGLVKPSETLSLTCTVSGYSITSGYYWNWIRQPPGKGLEWMGYISYDGSNNYNPSLKNRVTISRDTSKNQFSLKLSSVTAADTAVYYCARAYYGNYVGYFDVWGQGTTVTVSS

SEQ ID NO: 10 - protein, 121 aa, Artificial sequence
  heavy chain variable region of hAKB1 VH2
QVQLQESGPGLVKPSETLSLTCTVSGYSISSGYYWNWIRQPPGKGLEWMGYISYDGSNNYNPSLKNRVTISRDTSKNQFSLKLSSVTAADTAVYYCARAYYGNYVGYFDVWGQGTTVTVSS

SEQ ID NO: 11 - protein, 110 aa, Artificial sequence
  light chain variable region of hAKB1 VL1
DIQMTQSPSSLSASVGDRVTITCKASQSVSNDVAWYQQKPGKAPKLLIYYASNRYTGVPSRFSGSGYGTDFTFTISSLQPEDIATYYCQQDYSSPLTFGGGTKVEIKRTV

SEQ ID NO: 12 - protein, 110 aa, Artificial sequence
  light chain variable region of hAKB1 VL2
DIQMTQSPSSLSASVGDRVTITCKASQSVSNDVAWYQQKPGKAPKLLIYYASNRYTGVPSRFSGSGSGTDFTFTISSLQPEDIATYYCQQDYSSPLTFGGGTKVEIKRTV

SEQ ID NO: 13 - protein, 451 aa, Artificial sequence
  heavy chain of hAKB1-A without signal peptide
QVQLQESGPGLVKPSETLSLTCTVSGYSITSGYYWNWIRQPPGKGLEWMGYISYDGSNNYNPSLKNRVTISRDTSKNQFSLKLSSVTAADTAVYYCARAYYGNYVGYFDVWGQGTTVTVSSASTKGPSVFPLAPSSKSTSGGTAALGCLVKDYFPEPVTVSWNSGALTSGVHTFPAVLQSSGLYSLSSVVTVPSSSLGTQTYICNVNHKPSNTKVDKKVEPKSCDKTHTCPPCPAPEAAGGPSVFLFPPKPKDTLMISRTPEVTCVVVDVSHEDPEVKFNWYVDGVEVHNAKTKPREEQYNSTYRVVSVLTVLHQDWLNGKEYKCKVSNKALPAPIEKTISKAKGQPREPQVYTLPPSRDELTKNQVSLTCLVKGFYPSDIAVEWESNGQPENNYKTTPPVLDSDGSFFLYSKLTVDKSRWQQGNVFSCSVMHEALHNHYTQKSLSLSPGK

SEQ ID NO: 14 - protein, 451 aa, Artificial sequence
  heavy chain of hAKB1-B without signal peptide
QVQLQESGPGLVKPSETLSLTCTVSGYSISSGYYWNWIRQPPGKGLEWMGYISYDGSNNYNPSLKNRVTISRDTSKNQFSLKLSSVTAADTAVYYCARAYYGNYVGYFDVWGQGTTVTVSSASTKGPSVFPLAPSSKSTSGGTAALGCLVKDYFPEPVTVSWNSGALTSGVHTFPAVLQSSGLYSLSSVVTVPSSSLGTQTYICNVNHKPSNTKVDKKVEPKSCDKTHTCPPCPAPEAAGGPSVFLFPPKPKDTLMISRTPEVTCVVVDVSHEDPEVKFNWYVDGVEVHNAKTKPREEQYNSTYRVVSVLTVLHQDWLNGKEYKCKVSNKALPAPIEKTISKAKGQPREPQVYTLPPSRDELTKNQVSLTCLVKGFYPSDIAVEWESNGQPENNYKTTPPVLDSDGSFFLYSKLTVDKSRWQQGNVFSCSVMHEALHNHYTQKSLSLSPGK

SEQ ID NO: 15 - protein, 214 aa, Artificial sequence
  light chain of hAKB1-A and hAKB1-B without signal peptide
DIQMTQSPSSLSASVGDRVTITCKASQSVSNDVAWYQQKPGKAPKLLIYYASNRYTGVPSRFSGSGYGTDFTFTISSLQPEDIATYYCQQDYSSPLTFGGGTKVEIKRTVAAPSVFIFPPSDEQLKSGTASVVCLLNNFYPREAKVQWKVDNALQSGNSQESVTEQDSKDSTYSLSSTLTLSKADYEKHKVYACEVTHQGLSSPVTKSFNRGEC

SEQ ID NO: 16 - protein, 469 aa, Artificial sequence
  heavy chain of hAKB1-A with signal peptide
MKVLSLLYLLTAIPGILSQVQLQESGPGLVKPSETLSLTCTVSGYSITSGYYWNWIRQPPGKGLEWMGYISYDGSNNYNPSLKNRVTISRDTSKNQFSLKLSSVTAADTAVYYCARAYYGNYVGYFDVWGQGTTVTVSSASTKGPSVFPLAPSSKSTSGGTAALGCLVKDYFPEPVTVSWNSGALTSGVHTFPAVLQSSGLYSLSSVVTVPSSSLGTQTYICNVNHKPSNTKVDKKVEPKSCDKTHTCPPCPAPEAAGGPSVFLFPPKPKDTLMISRTPEVTCVVVDVSHEDPEVKFNWYVDGVEVHNAKTKPREEQYNSTYRVVSVLTVLHQDWLNGKEYKCKVSNKALPAPIEKTISKAKGQPREPQVYTLPPSRDELTKNQVSLTCLVKGFYPSDIAVEWESNGQPENNYKTTPPVLDSDGSFFLYSKLTVDKSRWQQGNVFSCSVMHEALHNHYTQKSLSLSPGK

SEQ ID NO: 17 - protein, 469 aa, Artificial sequence
  heavy chain of hAKB1-B with signal peptide
MKVLSLLYLLTAIPGILSQVQLQESGPGLVKPSETLSLTCTVSGYSISSGYYWNWIRQPPGKGLEWMGYISYDGSNNYNPSLKNRVTISRDTSKNQFSLKLSSVTAADTAVYYCARAYYGNYVGYFDVWGQGTTVTVSSASTKGPSVFPLAPSSKSTSGGTAALGCLVKDYFPEPVTVSWNSGALTSGVHTFPAVLQSSGLYSLSSVVTVPSSSLGTQTYICNVNHKPSNTKVDKKVEPKSCDKTHTCPPCPAPEAAGGPSVFLFPPKPKDTLMISRTPEVTCVVVDVSHEDPEVKFNWYVDGVEVHNAKTKPREEQYNSTYRVVSVLTVLHQDWLNGKEYKCKVSNKALPAPIEKTISKAKGQPREPQVYTLPPSRDELTKNQVSLTCLVKGFYPSDIAVEWESNGQPENNYKTTPPVLDSDGSFFLYSKLTVDKSRWQQGNVFSCSVMHEALHNHYTQKSLSLSPGK

SEQ ID NO: 18 - protein, 234 aa, Artificial sequence
  light chain of hAKB1-A and hAKB1-B with signal peptide
MKSQTQVFVFLLLCVSGAHGDIQMTQSPSSLSASVGDRVTITCKASQSVSNDVAWYQQKPGKAPKLLIYYASNRYTGVPSRFSGSGYGTDFTFTISSLQPEDIATYYCQQDYSSPLTFGGGTKVEIKRTVAAPSVFIFPPSDEQLKSGTASVVCLLNNFYPREAKVQWKVDNALQSGNSQESVTEQDSKDSTYSLSSTLTLSKADYEKHKVYACEVTHQGLSSPVTKSFNRGEC

SEQ ID NO: 19 - DNA, 1410 bp, Artificial sequence
  coding region of heavy chain of hAKB1-A
atgaaagtgttgagtctgttgtacctgttgacagccattcctggtatcctgtctcaagttcagcttcaggagtcaggacctggcctcgtgaaaccttctgagactctgtctctcacctgcactgtcagtggctactccatcaccagtggttattactggaactggatccggcagcctccaggaaaaggactggaatggatgggctacatcagctacgacggcagcaataactacaacccaagtctcaagaatcgagtcaccatcagtcgtgacacatctaagaaccagttttccctgaagttgagttctgtgactgctgccgacacagctgtgtattactgtgcaagggcctactatgggaactatgtgggctacttcgatgtctggggccaagggaccactgtcaccgtctcctcagcctccaccaagggcccatcggtcttccccctggcaccctcctccaagagcacctctgggggcacagcggccctgggctgcctggtcaaggactacttccccgaaccggtgacggtgtcgtggaactcaggcgccctgaccagcggcgtgcacaccttcccggctgtcctacagtcctcaggactctactccctcagcagcgtggtgaccgtgccctccagcagcttgggcacccagacctacatctgcaacgtgaatcacaagcccagcaacaccaaggtggacaagaaagttgagcccaaatcttgtgacaaaactcacacatgcccaccgtgcccagcacctgaagctgctggaggaccgtcagtcttcctcttccccccaaaacccaaggacaccctcatgatctcccggacccctgaggtcacatgcgtggtggtggacgtgagccacgaagaccctgaggtcaagttcaactggtacgtggacggcgtggaggtgcataatgccaagacaaagccgcgggaggagcagtacaacagcacgtaccgtgtggtcagcgtcctcaccgtcctgcaccaggactggctgaatggcaaggagtacaagtgcaaggtctccaacaaagccctcccagcccccatcgagaaaaccatctccaaagccaaagggcagccccgagaaccacaggtgtacaccctgcccccatcccgggatgagctgaccaagaaccaggtcagcctgacctgcctggtcaaaggcttctatcccagcgacatcgccgtggagtgggagagcaatgggcagccggagaacaactacaagaccacgcctcccgtgctggactccgacggctccttcttcctctacagcaagctcaccgtggacaagagcaggtggcagcaggggaacgtcttctcatgctccgtgatgcatgaggctctgcacaaccactacacgcagaagagcctctccctgtctccgggtaaatga

SEQ ID NO: 20 - DNA, 1410 bp, Artificial sequence
  coding region of heavy chain of hAKB1-B
atgaaagtgttgagtctgttgtacctgttgacagccattcctggtatcctgtctcaagttcagcttcaggagtcaggacctggcctcgtgaaaccttctgagactctgtctctcacctgcactgtcagtggctactccatcagcagtggttattactggaactggatccggcagcctccaggaaaaggactggaatggatgggctacatcagctacgacggcagcaataactacaacccaagtctcaagaatcgagtcaccatcagtcgtgacacatctaagaaccagttttccctgaagttgagttctgtgactgctgccgacacagctgtgtattactgtgcaagggcctactatgggaactatgtgggctacttcgatgtctggggccaagggaccactgtcaccgtctcctcagcctccaccaagggcccatcggtcttccccctggcaccctcctccaagagcacctctgggggcacagcggccctgggctgcctggtcaaggactacttccccgaaccggtgacggtgtcgtggaactcaggcgccctgaccagcggcgtgcacaccttcccggctgtcctacagtcctcaggactctactccctcagcagcgtggtgaccgtgccctccagcagcttgggcacccagacctacatctgcaacgtgaatcacaagcccagcaacaccaaggtggacaagaaagttgagcccaaatcttgtgacaaaactcacacatgcccaccgtgcccagcacctgaagctgctggaggaccgtcagtcttcctcttccccccaaaacccaaggacaccctcatgatctcccggacccctgaggtcacatgcgtggtggtggacgtgagccacgaagaccctgaggtcaagttcaactggtacgtggacggcgtggaggtgcataatgccaagacaaagccgcgggaggagcagtacaacagcacgtaccgtgtggtcagcgtcctcaccgtcctgcaccaggactggctgaatggcaaggagtacaagtgcaaggtctccaacaaagccctcccagcccccatcgagaaaaccatctccaaagccaaagggcagccccgagaaccacaggtgtacaccctgcccccatcccgggatgagctgaccaagaaccaggtcagcctgacctgcctggtcaaaggcttctatcccagcgacatcgccgtggagtgggagagcaatgggcagccggagaacaactacaagaccacgcctcccgtgctggactccgacggctccttcttcctctacagcaagctcaccgtggacaagagcaggtggcagcaggggaacgtcttctcatgctccgtgatgcatgaggctctgcacaaccactacacgcagaagagcctctccctgtctccgggtaaatga

SEQ ID NO: 21 - DNA, 705 bp, Artificial sequence
  coding region of light chain of hAKB1-A and hAKB1-B
atgaagtcacagacccaagtcttcgtgtttctgctgctctgtgtgtctggagctcatggggatattcagatgacccagagtcccagctccctgtctgcatcagtgggagacagggttaccatcacctgcaaggccagtcagagcgtctccaatgatgtcgcttggtaccaacagaagccagggaaggctcctaaactgctgatctactatgcatccaatcgctacactggagtccctagtcgcttcagtggcagtggatatgggaccgatttcactttcaccatcagcagtctgcagcctgaagacatcgcaacttattactgtcagcaggattatagctctccactcactttcggaggagggaccaaagtcgagatcaaacgaactgtggctgcaccatctgtcttcatcttcccgccatctgatgagcagttgaaatctggaactgcctctgttgtgtgcctgctgaataacttctatcccagagaggccaaagtacagtggaaggtggataacgccctccaatcgggtaactcccaggagagtgtcacagagcaggacagcaaggacagcacctacagcctcagcagcaccctgacgctgagcaaagcagactacgagaaacacaaagtctacgcctgcgaagtcacccatcagggcctgagctcgcccgtcacaaagagcttcaacaggggagagtgttag

SEQ ID NO: 22 - protein, 451 aa, Artificial sequence; identical to SEQ ID NO: 14
  heavy chain of hTKB1 without signal peptide

SEQ ID NO: 23 - protein, 214 aa, Artificial sequence; identical to SEQ ID NO: 15
  light chain of hTKB1 without signal peptide

SEQ ID NO: 24 - protein, 470 aa, Artificial sequence
  heavy chain of hTKB1 with signal peptide
MKHLWFFLLLVAAPRWVLSQVQLQESGPGLVKPSETLSLTCTVSGYSISSGYYWNWIRQPPGKGLEWMGYISYDGSNNYNPSLKNRVTISRDTSKNQFSLKLSSVTAADTAVYYCARAYYGNYVGYFDVWGQGTTVTVSSASTKGPSVFPLAPSSKSTSGGTAALGCLVKDYFPEPVTVSWNSGALTSGVHTFPAVLQSSGLYSLSSVVTVPSSSLGTQTYICNVNHKPSNTKVDKKVEPKSCDKTHTCPPCPAPEAAGGPSVFLFPPKPKDTLMISRTPEVTCVVVDVSHEDPEVKFNWYVDGVEVHNAKTKPREEQYNSTYRVVSVLTVLHQDWLNGKEYKCKVSNKALPAPIEKTISKAKGQPREPQVYTLPPSRDELTKNQVSLTCLVKGFYPSDIAVEWESNGQPENNYKTTPPVLDSDGSFFLYSKLTVDKSRWQQGNVFSCSVMHEALHNHYTQKSLSLSPGK

SEQ ID NO: 25 - protein, 236 aa, Artificial sequence
  light chain of hTKB1 with signal peptide
MDMRVPAQLLGLLLLWLRGARCDIQMTQSPSSLSASVGDRVTITCKASQSVSNDVAWYQQKPGKAPKLLIYYASNRYTGVPSRFSGSGYGTDFTFTISSLQPEDIATYYCQQDYSSPLTFGGGTKVEIKRTVAAPSVFIFPPSDEQLKSGTASVVCLLNNFYPREAKVQWKVDNALQSGNSQESVTEQDSKDSTYSLSSTLTLSKADYEKHKVYACEVTHQGLSSPVTKSFNRGEC

SEQ ID NO: 26 - DNA, 1416 bp, Artificial sequence
  coding region of heavy chain of hTKB1
atgaaacacctgtggttcttcctcctcctggtggcagctcccagatgggtcctgtcccaagttcagctgcaagaatccggacccggactggtgaagccctccgagactttatctttaacttgtaccgtgagcggctactccatctcctccggctactactggaactggattcgtcagcctcccggcaagggtttagaatggatgggctacatctcctacgacggctccaacaactacaacccctctttaaagaatcgtgtgaccatctctcgtgacacctccaagaaccagttctctttaaagctgtcctccgtgacagccgccgataccgccgtgtactactgcgctcgtgcctactacggcaactacgtgggctacttcgacgtgtggggccaaggtaccaccgtgacagtctcctccgctagcaccaagggcccatcggtcttccccctggcaccctcctccaagagcacctctgggggcacagcggccctgggctgcctggtcaaggactacttccccgaaccggtgacggtgtcgtggaactcaggcgccctgaccagcggcgtgcacaccttcccggccgtcctacagtcctcaggactctactccctcagcagcgtggtgaccgtgccctccagcagcttgggcacccagacctacatctgcaacgtgaatcacaagcccagcaacaccaaggtggacaagaaggttgagcccaaatcttgtgacaaaactcacacatgcccaccgtgcccagcacctgaagcagccgggggaccgtcagtcttcctcttccccccaaaacccaaggacaccctcatgatctcccggacccctgaggtcacatgcgtggtggtggacgtgagccacgaagaccctgaggtcaagttcaactggtacgtggacggcgtggaggtgcataatgccaagacaaagccgcgggaggagcagtacaacagcacgtaccgtgtggtcagcgtcctcaccgtcctgcaccaggactggctgaatggcaaggagtacaagtgcaaggtctccaacaaagccctcccagcccccatcgagaaaaccatctccaaagccaaagggcagccccgagaaccacaggtgtacaccctgcccccatcccgggacgagctgaccaagaaccaggtcagcctgacctgcctggtcaaaggcttctatcccagcgacatcgccgtggagtgggagagcaatgggcagccggagaacaactacaagaccacgcctcccgtgctggactccgacggctccttcttcctctacagcaagctcaccgtggacaagagcaggtggcagcaggggaacgtcttctcatgctccgtgatgcatgaggctctgcacaaccactacacgcagaagagcctctccctgtctccgggtaaatgatga

SEQ ID NO: 27 - DNA, 714 bp, Artificial sequence
  coding region of light chain of hTKB1
atggacatgagggtccccgctcagctcctggggctcctgctactctggctccgaggtgccagatgtgacatccagatgacccagtccccttcctctttaagcgcttccgtgggcgatcgtgtgaccatcacttgtaaggcctcccagtccgtgtccaacgacgtggcttggtaccagcagaagcccggcaaggcccccaagctgctgatctactacgcctccaatcgttacaccggcgtgccttctcgtttttccggctccggctacggcaccgacttcaccttcaccatctcctctttacagcccgaggacatcgccacctactactgccagcaagattactcctcccctctgacctttggcggcggcaccaaggtggagatcaagcgtacggtggctgcaccatctgtcttcatcttcccgccatctgatgagcagttgaaatctggaactgcctctgttgtgtgcctgctgaataacttctatcccagagaggccaaagtacagtggaaggtggataacgccctccaatcgggtaactcccaggagagtgtcacagagcaggacagcaaggacagcacctacagcctcagcagcaccctgacgctgagcaaagcagactacgagaaacacaaagtctacgcctgcgaagtcacccatcagggcctgagctcgcccgtcacaaagagcttcaacaggggagagtgttgatga

SEQ ID NO: 28 - protein, 18 aa, Artificial sequence
  signal peptide of heavy chain of hAKB1-A
MKVLSLLYLLTAIPGILS

SEQ ID NO: 29 - protein, 18 aa, Artificial sequence
  signal peptide of heavy chain of hAKB1-B
MKVLSLLYLLTAIPGILS

SEQ ID NO: 30 - protein, 20 aa, Artificial sequence
  signal peptide of light chain of hAKB1-A and hAKB1-B
MKSQTQVFVFLLLCVSGAHG

SEQ ID NO: 31 - protein, 19 aa, Artificial sequence
  signal peptide of heavy chain of hTKB1
MKHLWFFLLLVAAPRWVLS

SEQ ID NO: 32 - protein, 22 aa, Artificial sequence
  signal peptide of light chain of hTKB1
MDMRVPAQLLGLLLLWLRGARC

SEQ ID NO: 33 - DNA, 21 bp, Artificial sequence
  Gapdh forward primer
cttcaccaccatggagaaggc

SEQ ID NO: 34 - DNA, 21 bp, Artificial sequence
  Gapdh reverse primer
ggcatggactgtggtcatgag

SEQ ID NO: 35 - DNA, 22 bp, Artificial sequence
  Ifng forward primer
accagagcatccaaaagagtgt

SEQ ID NO: 36 - DNA, 20 bp, Artificial sequence
  Ifng reverse primer
ttagctgctggcgacagttc

SEQ ID NO: 37 - DNA, 21 bp, Artificial sequence
  Tnfa forward primer
cagcctcttctccttcctgat

SEQ ID NO: 38 - DNA, 20 bp, Artificial sequence
  Tnfa reverse primer
gccagagggctgattagaga